European Patent Specification EP 3 415 628 B1, published March 8, 2023. Title: Recombinant Variant Microorganism Having a Producing Ability of Malonic Acid and Method for Preparing Malonic Acid Using the Same. Applicant: KOREA ADVANCED INSTITUTE OF SCIENCE AND TECHNOLOGY HANWHA CHEMICAL CORPORATION. The sequence listing filed with the application follows.

SEQUENCE LISTING (14 sequences)

SEQ ID NO: 1 - DNA, 37 bp, Artificial Sequence
  ppc F
agacagcctgcaggttagccggtattacgcatacctg

SEQ ID NO: 2 - DNA, 48 bp, Artificial Sequence
  ppc R
agacagcctgcaggacaggaaacagaccatgaacgaacaatattccgc

SEQ ID NO: 3 - DNA, 33 bp, Artificial Sequence
  pa0132 F
agacagtctagagaaagcccgaggatcgaacga

SEQ ID NO: 4 - DNA, 33 bp, Artificial Sequence
  pa0132 R
agacagcctgcaggtcaggcgatgccgttgagc

SEQ ID NO: 5 - DNA, 51 bp, Artificial Sequence
  pa4123 F
agacaggagctcacaggaaacagaccatgatcaaacactggatcaatggcc

SEQ ID NO: 6 - DNA, 31 bp, Artificial Sequence
  pa4123 R
agacagtctagactacacgccccagcggggg

SEQ ID NO: 7 - DNA, 51 bp, Artificial Sequence
  yneI F
agacaggagctcacaggaaacagaccatgaccattactccggcaactcatg

SEQ ID NO: 8 - DNA, 35 bp, Artificial Sequence
  yneI R
agacagtctagatcagatccggtctttccacaccg

SEQ ID NO: 9 - DNA, 35 bp, Artificial Sequence
  p100
ttgacggctagctcagtcctaggtacagtgctagc

SEQ ID NO: 10 - DNA, 1461 bp, Pseudomonas aeruginosa
atgatcaaacactggatcaatggccgcgaggtcgaaagcaaggacgtcttcgagaactacaacccggccaccggcgagctgatcggcgaggtcgccagcggcggcgcggcggaaatcgacgcggcggtggcggcggcccgggaagccttcccgaaatgggccaataccccggccaaggagcgcgcgcgcctgatgcgccggctcggcgagctgatcgaccggaacgtgccgcacctggcggaacttgagaccctcgacaccggcctgccgatccaccagacgaagaacgtgctgatcccgcgcgcctcgcacaacttcgagttcttcgccgaagtctgcacgcggatgaacgggcacagctatccggtcgacgaccagatgctcaactacaccctgtaccagccggtaggcgtctgcggcctggtctcgccgtggaacgtaccgttcatgaccgccacctggaagaccgcgccgtgcctggcgctgggcaacacggcggtgctgaagatgtccgagctgtcgccgctgaccgccaacgagctgggccgcctggtgcacgaggcgggcattccgccgggggtgttcaacgtggtccagggctacggcgccagcgccggcgacgcgctggttcgccaccgcgacgtgcgcgcggtgtccttcaccggcggcaccgccaccgggcgacggatcatggaggcggccgggatcaagaaatactcgatggaactgggcggcaagtcgccggtgctggtcttcgaagacgccgacctcgagcgggcgctggacgccgctctgttcaccatcttctcgctgaacggcgagcgctgcaccgccggcagtcgcatcttcgtccaggaaagcgtctacccgcagttcgtcgccgagttcgccgcgcgcgccaggcgcctgatcgtcggcgatccgcaggacccgaagacccaggtcggctcgatgatcacccaggcccactacgacaaggtcaccggctacatccgcatcggcctcgaggaaggcgccaccctggtggccggcggcctggagcgtccggccggcctgccggcgcacctgagcaaggggcagttcatccagcccacggtgttcgccgacgtggacaaccgcatgcgcatcgcccaggaggagatcttcggcccggtggtctgcctgatcccgttcaaggacgaagccgaggcgctgcgcctggccaacgacgtggaatacggcctggcctcctacatctggacccaggacatcggcaaggcccatcgcctggcacgcggcatcgaggccgggatggtcttcatcaacagccagaacgtgcgcgacctgcgccagccgttcggcggggtgaaggcctcgggcaccggacgcgaaggcggggaatacagcttcgaggtattcgccgagatcaagaacgtgtgtatatccatgggcagccatcacatcccccgctggggcgtgtag

SEQ ID NO: 11 - protein, 486 aa, Pseudomonas aeruginosa
MIKHWINGREVESKDVFENYNPATGELIGEVASGGAAEIDAAVAAAREAFPKWANTPAKERARLMRRLGELIDRNVPHLAELETLDTGLPIHQTKNVLIPRASHNFEFFAEVCTRMNGHSYPVDDQMLNYTLYQPVGVCGLVSPWNVPFMTATWKTAPCLALGNTAVLKMSELSPLTANELGRLVHEAGIPPGVFNVVQGYGASAGDALVRHRDVRAVSFTGGTATGRRIMEAAGIKKYSMELGGKSPVLVFEDADLERALDAALFTIFSLNGERCTAGSRIFVQESVYPQFVAEFAARARRLIVGDPQDPKTQVGSMITQAHYDKVTGYIRIGLEEGATLVAGGLERPAGLPAHLSKGQFIQPTVFADVDNRMRIAQEEIFGPVVCLIPFKDEAEALRLANDVEYGLASYIWTQDIGKAHRLARGIEAGMVFINSQNVRDLRQPFGGVKASGTGREGGEYSFEVFAEIKNVCISMGSHHIPRWGV

SEQ ID NO: 12 - DNA, 1389 bp, Escherichia coli
atgaccattactccggcaactcatgcaatttcgataaatcctgccacgggtgaacaactttctgtgctgccgtgggctggcgctgacgatatcgaaaacgcacttcagctggcggcagcaggctttcgcgactggcgcgagacaaatatagattatcgtgctgaaaaactgcgtgatatcggtaaggctctgcgcgctcgtagcgaagaaatggcgcaaatgatcacccgcgaaatgggcaaaccaatcaaccaggcgcgcgctgaagtggcgaaatcggcgaatttgtgtgactggtatgcagaacatggtccggcaatgctgaaggcggaacctacgctggtggaaaatcagcaggcggttattgagtatcgaccgttggggacgattctggcgattatgccgtggaattttccgttatggcaggtgatgcgtggcgctgttcccatcattcttgcaggtaacggctacttacttaaacatgcgccgaatgtgatgggctgtgcacagctcattgcccaggtgtttaaagatgcgggtatcccacaaggcgtatatggctggctgaatgccgacaacgacggtgtcagtcagatgattaaagactcgcgcattgctgctgtcacggtgaccggaagtgttcgtgcgggagcggctattggcgcacaggctggagcggcactgaaaaaatgcgtactggaactgggcggttcggatccgtttattgtgcttaacgatgccgatctggaactggcggtgaaagcggcggtagccggacgttatcagaataccggacaggtatgtgcagcggcaaaacgctttattatcgaagagggaattgcttcggcatttaccgaacgttttgtggcagctgcggcagccttgaaaatgggcgatccccgtgacgaagagaacgctctcggaccaatggctcgttttgatttacgtgatgagctgcatcatcaggtggagaaaaccctggcgcagggtgcgcgtttgttactgggcggggaaaagatggctggggcaggtaactactatccgccaacggttctggcgaatgttaccccagaaatgaccgcgtttcgggaagaaatgtttggccccgttgcggcaatcaccattgcgaaagatgcagaacatgcactggaactggctaatgatagtgagttcggcctttcagcgaccatttttaccactgacgaaacacaggccagacagatggcggcacgtctggaatgcggtggggtgtttatcaatggttattgtgccagcgacgcgcgagtggcctttggtggcgtgaaaaagagtggctttggtcgtgagctttcccatttcggcttacacgaattctgtaatatccagacggtgtggaaagaccggatctga

SEQ ID NO: 13 - protein, 462 aa, Escherichia coli
MTITPATHAISINPATGEQLSVLPWAGADDIENALQLAAAGFRDWRETNIDYRAEKLRDIGKALRARSEEMAQMITREMGKPINQARAEVAKSANLCDWYAEHGPAMLKAEPTLVENQQAVIEYRPLGTILAIMPWNFPLWQVMRGAVPIILAGNGYLLKHAPNVMGCAQLIAQVFKDAGIPQGVYGWLNADNDGVSQMIKDSRIAAVTVTGSVRAGAAIGAQAGAALKKCVLELGGSDPFIVLNDADLELAVKAAVAGRYQNTGQVCAAAKRFIIEEGIASAFTERFVAAAAALKMGDPRDEENALGPMARFDLRDELHHQVEKTLAQGARLLLGGEKMAGAGNYYPPTVLANVTPEMTAFREEMFGPVAAITIAKDAEHALELANDSEFGLSATIFTTDETQARQMAARLECGGVFINGYCASDARVAFGGVKKSGFGRELSHFGLHEFCNIQTVWKDRI

SEQ ID NO: 14 - DNA, 1347 bp, Pseudomonas aeruginosa
atgaaccagccgctcaacgtggccccgccggtttccagcgaactcaacctgcgcgcccactggatgcccttctccgccaaccgcaacttccagaaggacccgcggatcatcgtcgccgccgaaggcagctggctgaccgacgacaagggccgcaaggtctacgacagcctgtccggcctgtggacctgcggcgccggccactcgcgcaaggaaatccaggaggcggtggctcgccagctcggcaccctcgactactcgccgggcttccagtacggccatccgctgtccttccagttggccgagaagatcgccgggttgctgccaggcgaactgaaccacgtgttcttcaccggttccggctccgagtgcgccgacacctcgatcaagatggcccgcgcctactggcgcctgaaaggccagccgcagaagaccaagctgatcggccgcgcccgcggctaccacggggtcaacgtcgccggcaccagcctcggcgggatcggtggcaaccgcaagatgttcggccagctgatggacgtcgaccatctgccgcacacccttcaaccgggcatggcgttcacccgcgggatggcccagaccggcggcgtcgagctggccaacgagctgctcaagctgatcgaactgcacgacgcctcgaacatcgccgcggtgatcgtcgagccgatgtccggctccgccggcgtactggtaccgccggtcggctacctgcagcgcctgcgcgagatctgcgaccagcacaacatcctgctgatcttcgacgaggtgatcaccgccttcggccgcctgggcacctacagcggcgccgagtacttcggcgtcaccccggacctgatgaacgtcgccaagcaggtcaccaacggcgccgtgccgatgggcgcggtgatcgccagcagcgagatctacgacaccttcatgaaccaggcgctgcccgagcacgcggtggagttcagccacggctacacctactccgcgcacccggtcgcctgcgccgccggcctcgccgcgctggacatcctggccagggacaacctggtgcagcagtccgccgagctggcgccgcacttcgagaagggcctgcacggcctgcaaggcgcgaagaacgtcatcgacatccgcaactgcggcctggccggcgcgatccagatcgccccgcgcgacggcgatccgaccgtgcgtccgttcgaggccggcatgaagctctggcaacagggtttctacgtgcgcttcggcggcgataccctgcaattcggcccgaccttcaacgccaggccggaagagctggaccgcctgttcgacgcggtcggcgaagcgctcaacggcatcgcctga